European Patent Application EP 4 786 469 A1, published August 5, 2026. Title: 含三氮唑基化合物、制备方法及用途. Applicant: 上海拓界生物医药科技有限公司. Application WO. The sequence listing filed with the application follows.

SEQUENCE LISTING (56 sequences)

SEQ ID NO: 1 - RNA, 21 nt, Synthetic Construct
  source 1..21: mol_type = other RNA; note = unmodified sense strand; note (original language) = 未修饰的正义链; organism (original language) = 合成构建体
  modified_base 17: mod_base = OTHER; note = n is a hypoxanthine 2'-OMe riboside; note (original language) = n为次黄嘌呤2'-OMe核糖核苷
ccacatgatccatgctnagta

SEQ ID NO: 2 - RNA, 21 nt, Synthetic Construct
  source 1..21: mol_type = other RNA; note = unmodified antisense strand; note (original language) = 未修饰的正反义链; organism (original language) = 合成构建体
tactcagcatggatcatgtgg

SEQ ID NO: 3 - RNA, 21 nt, Synthetic Construct
  source 1..21: mol_type = other RNA; note = unmodified sense strand; note (original language) = 未修饰的正义链; organism (original language) = 合成构建体
gtgctttaactacaatataca

SEQ ID NO: 4 - RNA, 23 nt, Synthetic Construct
  source 1..23: mol_type = other RNA; note = unmodified antisense strand; note (original language) = 未修饰的反义链; organism (original language) = 合成构建体
tgtatattgtagttaaagcacat

SEQ ID NO: 5 - RNA, 21 nt, Synthetic Construct
  source 1..21: mol_type = other RNA; note = unmodified sense strand; note (original language) = 未修饰的正义链; organism (original language) = 合成构建体
ccggtcccaggttatgacaca

SEQ ID NO: 6 - RNA, 23 nt, Synthetic Construct
  source 1..23: mol_type = other RNA; note = unmodified antisense strand; note (original language) = 未修饰的反义链; organism (original language) = 合成构建体
tgtgtcataacctgggaccggat

SEQ ID NO: 7 - RNA, 22 nt, Synthetic Construct
  source 1..22: mol_type = other RNA; note = modified sense strand; note (original language) = 经修饰的正义链
  modified_base 1..8: mod_base = OTHER; note = modified with 2'-methoxy; note (original language) = 2'-甲氧基修饰的
  modified_base 9..11: mod_base = OTHER; note = modified with 2'-Fluoro; note (original language) = 2'-氟代修饰的
  modified_base 12..21: mod_base = OTHER; note = modified with 2'-methoxy; note (original language) = 2'-甲氧基修饰的
  modified_base 17: mod_base = OTHER; note = n is a hypoxanthine 2'-OMe riboside; note (original language) = n为次黄嘌呤2'-OMe核糖核苷
  modified_base 22: mod_base = OTHER; note = n is a reverse reverse nucleotide without base modification; note (original language) = n为反向无碱基修饰的核苷
  modified_base 1..2: mod_base = OTHER; note = two adjacent nucleosides are linked by phosphorothioate diester groups; note (original language) = 相邻的两个核苷之间为硫代磷酸二酯基连接
  modified_base 21..22: mod_base = OTHER; note = two adjacent nucleosides are linked by phosphorothioate diester groups; note (original language) = 相邻的两个核苷之间为硫代磷酸二酯基连接
  modified_base 1: mod_base = OTHER; note = the 5' end is conjugated with the II-1; note (original language) = 5'端与II-1缀合
ccacatgatccatgctnagtan

SEQ ID NO: 8 - RNA, 22 nt, Synthetic Construct
  source 1..22: mol_type = other RNA; note = modified sense strand; note (original language) = 经修饰的正义链; organism (original language) = 合成构建体
  modified_base 17: mod_base = OTHER; note = n is a hypoxanthine 2'-OMe riboside; note (original language) = n为次黄嘌呤2'-OMe核糖核苷
  modified_base 22: mod_base = OTHER; note = n is a reverse reverse nucleotide without base modification; note (original language) = n为反向无碱基修饰的核苷
  modified_base 1..8: mod_base = OTHER; note = modified with 2'-methoxy; note (original language) = 2'-甲氧基修饰的
  modified_base 9..11: mod_base = OTHER; note = modified with 2'-Fluoro; note (original language) = 2'-氟代修饰的
  modified_base 12..21: mod_base = OTHER; note = modified with 2'-methoxy; note (original language) = 2'-甲氧基修饰的
  modified_base 1..2: mod_base = OTHER; note = two adjacent nucleosides are linked by phosphorothioate diester groups; note (original language) = 相邻的两个核苷之间为硫代磷酸二酯基连接
  modified_base 21..22: mod_base = OTHER; note = two adjacent nucleosides are linked by phosphorothioate diester groups; note (original language) = 相邻的两个核苷之间为硫代磷酸二酯基连接
  modified_base 1: mod_base = OTHER; note = the 5' end is conjugated with the II-5; note (original language) = 5'端与II-5缀合
ccacatgatccatgctnagtan

SEQ ID NO: 9 - RNA, 22 nt, Synthetic Construct
  source 1..22: mol_type = other RNA; note = modified sense strand; note (original language) = 经修饰的正义链
  modified_base 17: mod_base = OTHER; note = n is a hypoxanthine 2'-OMe riboside; note (original language) = n为次黄嘌呤2'-OMe核糖核苷
  modified_base 22: mod_base = OTHER; note = n is a reverse reverse nucleotide without base modification; note (original language) = n为反向无碱基修饰的核苷
  modified_base 1..8: mod_base = OTHER; note = modified with 2'-methoxy; note (original language) = 2'-甲氧基修饰的
  modified_base 9..11: mod_base = OTHER; note = modified with 2'-Fluoro; note (original language) = 2'-氟代修饰的
  modified_base 12..21: mod_base = OTHER; note = modified with 2'-methoxy; note (original language) = 2'-甲氧基修饰的
  modified_base 1..2: mod_base = OTHER; note = two adjacent nucleosides are linked by phosphorothioate diester groups; note (original language) = 相邻的两个核苷之间为硫代磷酸二酯基连接
  modified_base 21..22: mod_base = OTHER; note = two adjacent nucleosides are linked by phosphorothioate diester groups; note (original language) = 相邻的两个核苷之间为硫代磷酸二酯基连接
  modified_base 1: mod_base = OTHER; note = the 5' end is conjugated with the II-3; note (original language) = 5'端与II-3缀合
ccacatgatccatgctnagtan

SEQ ID NO: 10 - RNA, 22 nt, Synthetic Construct
  source 1..22: mol_type = other RNA; note = modified sense strand; note (original language) = 经修饰的正义链; organism (original language) = 合成构建体
  modified_base 17: mod_base = OTHER; note = n is a hypoxanthine 2'-OMe riboside; note (original language) = n为次黄嘌呤2'-OMe核糖核苷
  modified_base 22: mod_base = OTHER; note = n is a reverse reverse nucleotide without base modification; note (original language) = n为反向无碱基修饰的核苷
  modified_base 1..8: mod_base = OTHER; note = modified with 2'-methoxy; note (original language) = 2'-甲氧基修饰的
  modified_base 9..11: mod_base = OTHER; note = modified with 2'-Fluoro; note (original language) = 2'-氟代修饰的
  modified_base 12..21: mod_base = OTHER; note = modified with 2'-methoxy; note (original language) = 2'-甲氧基修饰的
  modified_base 1..2: mod_base = OTHER; note = two adjacent nucleosides are linked by phosphorothioate diester groups; note (original language) = 相邻的两个核苷之间为硫代磷酸二酯基连接
  modified_base 21..22: mod_base = OTHER; note = two adjacent nucleosides are linked by phosphorothioate diester groups; note (original language) = 相邻的两个核苷之间为硫代磷酸二酯基连接
  modified_base 1: mod_base = OTHER; note = the 5' end is conjugated with the II-2; note (original language) = 5'端与II-2缀合
ccacatgatccatgctnagtan

SEQ ID NO: 11 - RNA, 22 nt, Synthetic Construct
  source 1..22: mol_type = other RNA; note = modified sense strand; note (original language) = 经修饰的正义链; organism (original language) = 合成构建体
  modified_base 17: mod_base = OTHER; note = n is a hypoxanthine 2'-OMe riboside; note (original language) = n为次黄嘌呤2'-OMe核糖核苷
  modified_base 22: mod_base = OTHER; note = n is a reverse reverse nucleotide without base modification; note (original language) = n为反向无碱基修饰的核苷
  modified_base 1..8: mod_base = OTHER; note = modified with 2'-methoxy; note (original language) = 2'-甲氧基修饰的
  modified_base 9..11: mod_base = OTHER; note = modified with 2'-Fluoro; note (original language) = 2'-氟代修饰的
  modified_base 12..21: mod_base = OTHER; note = modified with 2'-methoxy; note (original language) = 2'-甲氧基修饰的
  modified_base 1..2: mod_base = OTHER; note = two adjacent nucleosides are linked by phosphorothioate diester groups; note (original language) = 相邻的两个核苷之间为硫代磷酸二酯基连接
  modified_base 21..22: mod_base = OTHER; note = two adjacent nucleosides are linked by phosphorothioate diester groups; note (original language) = 相邻的两个核苷之间为硫代磷酸二酯基连接
  modified_base 1: mod_base = OTHER; note = the 5' end is conjugated with the TA14'; note (original language) = 5'端与TA14'缀合
ccacatgatccatgctnagtan

SEQ ID NO: 12 - RNA, 22 nt, Synthetic Construct
  source 1..22: mol_type = other RNA; note = modified sense strand; note (original language) = 经修饰的正义链; organism (original language) = 合成构建体
  modified_base 22: mod_base = OTHER; note = n is a reverse reverse nucleotide without base modification; note (original language) = n为反向无碱基修饰的核苷
  modified_base 1..6: mod_base = OTHER; note = modified with 2'-methoxy; note (original language) = 2'-甲氧基修饰的
  modified_base 7: mod_base = OTHER; note = modified with 2'-Fluoro; note (original language) = 2'-氟代修饰的
  modified_base 8: mod_base = OTHER; note = modified with 2'-methoxy; note (original language) = 2'-甲氧基修饰的
  modified_base 9..11: mod_base = OTHER; note = modified with 2'-Fluoro; note (original language) = 2'-氟代修饰的
  modified_base 12..21: mod_base = OTHER; note = modified with 2'-methoxy; note (original language) = 2'-甲氧基修饰的
  modified_base 1..3: mod_base = OTHER; note = two adjacent nucleosides are linked by phosphorothioate diester groups; note (original language) = 相邻的两个核苷之间为硫代磷酸二酯基连接
  modified_base 20..22: mod_base = OTHER; note = two adjacent nucleosides are linked by phosphorothioate diester groups; note (original language) = 相邻的两个核苷之间为硫代磷酸二酯基连接
  modified_base 1: mod_base = OTHER; note = the 5' end is conjugated with the II-3; note (original language) = 5'端与II-3缀合
gtgctttaactacaatatacan

SEQ ID NO: 13 - RNA, 22 nt, Synthetic Construct
  source 1..22: mol_type = other RNA; note = modified sense strand; note (original language) = 经修饰的正义链; organism (original language) = 合成构建体
  modified_base 22: mod_base = OTHER; note = n is a reverse reverse nucleotide without base modification; note (original language) = n为反向无碱基修饰的核苷
  modified_base 1..6: mod_base = OTHER; note = modified with 2'-methoxy; note (original language) = 2'-甲氧基修饰的
  modified_base 7: mod_base = OTHER; note = modified with 2'-Fluoro; note (original language) = 2'-氟代修饰的
  modified_base 8: mod_base = OTHER; note = modified with 2'-methoxy; note (original language) = 2'-甲氧基修饰的
  modified_base 9..11: mod_base = OTHER; note = modified with 2'-Fluoro; note (original language) = 2'-氟代修饰的
  modified_base 12..21: mod_base = OTHER; note = modified with 2'-methoxy; note (original language) = 2'-甲氧基修饰的
  modified_base 1..3: mod_base = OTHER; note = two adjacent nucleosides are linked by phosphorothioate diester groups; note (original language) = 相邻的两个核苷之间为硫代磷酸二酯基连接
  modified_base 20..22: mod_base = OTHER; note = two adjacent nucleosides are linked by phosphorothioate diester groups; note (original language) = 相邻的两个核苷之间为硫代磷酸二酯基连接
  modified_base 1: mod_base = OTHER; note = the 5' end is conjugated with the TA14'; note (original language) = 5'端与TA14'缀合
gtgctttaactacaatatacan

SEQ ID NO: 14 - RNA, 22 nt, Synthetic Construct
  source 1..22: mol_type = other RNA; note = modified sense strand; note (original language) = 经修饰的正义链; organism (original language) = 合成构建体
  modified_base 22: mod_base = OTHER; note = n is a reverse reverse nucleotide without base modification; note (original language) = n为反向无碱基修饰的核苷
  modified_base 1..6: mod_base = OTHER; note = modified with 2'-methoxy; note (original language) = 2'-甲氧基修饰的
  modified_base 7: mod_base = OTHER; note = modified with 2'-Fluoro; note (original language) = 2'-氟代修饰的
  modified_base 8: mod_base = OTHER; note = modified with 2'-methoxy; note (original language) = 2'-甲氧基修饰的
  modified_base 9..11: mod_base = OTHER; note = modified with 2'-Fluoro; note (original language) = 2'-氟代修饰的
  modified_base 12..21: mod_base = OTHER; note = modified with 2'-methoxy; note (original language) = 2'-甲氧基修饰的
  modified_base 1..2: mod_base = OTHER; note = two adjacent nucleosides are linked by phosphorothioate diester groups; note (original language) = 相邻的两个核苷之间为硫代磷酸二酯基连接
  modified_base 20..22: mod_base = OTHER; note = two adjacent nucleosides are linked by phosphorothioate diester groups; note (original language) = 相邻的两个核苷之间为硫代磷酸二酯基连接
  modified_base 1: mod_base = OTHER; note = the 5' end is conjugated with the II-2; note (original language) = 5'端与II-2缀合
gtgctttaactacaatatacan

SEQ ID NO: 15 - RNA, 22 nt, Synthetic Construct
  source 1..22: mol_type = other RNA; note = modified sense strand; note (original language) = 经修饰的正义链; organism (original language) = 合成构建体
  modified_base 22: mod_base = OTHER; note = n is a reverse reverse nucleotide without base modification; note (original language) = n为反向无碱基修饰的核苷
  modified_base 1..6: mod_base = OTHER; note = modified with 2'-methoxy; note (original language) = 2'-甲氧基修饰的
  modified_base 7: mod_base = OTHER; note = modified with 2'-Fluoro; note (original language) = 2'-氟代修饰的
  modified_base 8: mod_base = OTHER; note = modified with 2'-methoxy; note (original language) = 2'-甲氧基修饰的
  modified_base 9..11: mod_base = OTHER; note = modified with 2'-Fluoro; note (original language) = 2'-氟代修饰的
  modified_base 12..21: mod_base = OTHER; note = modified with 2'-methoxy; note (original language) = 2'-甲氧基修饰的
  modified_base 1..3: mod_base = OTHER; note = two adjacent nucleosides are linked by phosphorothioate diester groups; note (original language) = 相邻的两个核苷之间为硫代磷酸二酯基连接
  modified_base 20..22: mod_base = OTHER; note = two adjacent nucleosides are linked by phosphorothioate diester groups; note (original language) = 相邻的两个核苷之间为硫代磷酸二酯基连接
  modified_base 1: mod_base = OTHER; note = the 5' end is conjugated with the II-5; note (original language) = 5'端与II-5缀合
gtgctttaactacaatatacan

SEQ ID NO: 16 - RNA, 22 nt, Synthetic Construct
  source 1..22: mol_type = other RNA; note = modified sense strand; note (original language) = 经修饰的正义链; organism (original language) = 合成构建体
  modified_base 22: mod_base = OTHER; note = n is a reverse reverse nucleotide without base modification; note (original language) = n为反向无碱基修饰的核苷
  modified_base 1..6: mod_base = OTHER; note = modified with 2'-methoxy; note (original language) = 2'-甲氧基修饰的
  modified_base 7: mod_base = OTHER; note = modified with 2'-Fluoro; note (original language) = 2'-氟代修饰的
  modified_base 8: mod_base = OTHER; note = modified with 2'-methoxy; note (original language) = 2'-甲氧基修饰的
  modified_base 9..11: mod_base = OTHER; note = modified with 2'-Fluoro; note (original language) = 2'-氟代修饰的
  modified_base 12..21: mod_base = OTHER; note = modified with 2'-methoxy; note (original language) = 2'-甲氧基修饰的
  modified_base 1..3: mod_base = OTHER; note = two adjacent nucleosides are linked by phosphorothioate diester groups; note (original language) = 相邻的两个核苷之间为硫代磷酸二酯基连接
  modified_base 20..22: mod_base = OTHER; note = two adjacent nucleosides are linked by phosphorothioate diester groups; note (original language) = 相邻的两个核苷之间为硫代磷酸二酯基连接
  modified_base 1: mod_base = OTHER; note = the 5' end is conjugated with the II-3; note (original language) = 5'端与II-3缀合
ccggtcccaggttatgacacan

SEQ ID NO: 17 - RNA, 22 nt, Synthetic Construct
  source 1..22: mol_type = other RNA; note = modified sense strand; note (original language) = 经修饰的正义链; organism (original language) = 合成构建体
  modified_base 22: mod_base = OTHER; note = n is a reverse reverse nucleotide without base modification; note (original language) = n为反向无碱基修饰的核苷
  modified_base 1..6: mod_base = OTHER; note = modified with 2'-methoxy; note (original language) = 2'-甲氧基修饰的
  modified_base 7: mod_base = OTHER; note = modified with 2'-Fluoro; note (original language) = 2'-氟代修饰的
  modified_base 8: mod_base = OTHER; note = modified with 2'-methoxy; note (original language) = 2'-甲氧基修饰的
  modified_base 9..11: mod_base = OTHER; note = modified with 2'-Fluoro; note (original language) = 2'-氟代修饰的
  modified_base 12..21: mod_base = OTHER; note = modified with 2'-methoxy; note (original language) = 2'-甲氧基修饰的
  modified_base 1..3: mod_base = OTHER; note = two adjacent nucleosides are linked by phosphorothioate diester groups; note (original language) = 相邻的两个核苷之间为硫代磷酸二酯基连接
  modified_base 20..22: mod_base = OTHER; note = two adjacent nucleosides are linked by phosphorothioate diester groups; note (original language) = 相邻的两个核苷之间为硫代磷酸二酯基连接
  modified_base 1: mod_base = OTHER; note = the 5' end is conjugated with the TA14'; note (original language) = 5'端与TA14'缀合
ccggtcccaggttatgacacan

SEQ ID NO: 18 - RNA, 22 nt, Synthetic Construct
  source 1..22: mol_type = other RNA; note = modified sense strand; note (original language) = 经修饰的正义链; organism (original language) = 合成构建体
  modified_base 17: mod_base = OTHER; note = n is a hypoxanthine 2'-OMe riboside; note (original language) = n为次黄嘌呤2'-OMe核糖核苷
  modified_base 22: mod_base = OTHER; note = n is a reverse reverse nucleotide without base modification; note (original language) = n为反向无碱基修饰的核苷
  modified_base 1..8: mod_base = OTHER; note = modified with 2'-methoxy; note (original language) = 2'-甲氧基修饰的
  modified_base 9..11: mod_base = OTHER; note = modified with 2'-Fluoro; note (original language) = 2'-氟代修饰的
  modified_base 12..21: mod_base = OTHER; note = modified with 2'-methoxy; note (original language) = 2'-甲氧基修饰的
  modified_base 1..2: mod_base = OTHER; note = two adjacent nucleosides are linked by phosphorothioate diester groups; note (original language) = 相邻的两个核苷之间为硫代磷酸二酯基连接
  modified_base 21..22: mod_base = OTHER; note = two adjacent nucleosides are linked by phosphorothioate diester groups; note (original language) = 相邻的两个核苷之间为硫代磷酸二酯基连接
  modified_base 1: mod_base = OTHER; note = the 5' end is conjugated with the targeting ligand III-1; note (original language) = 5'端与靶向配体III-1缀合
ccacatgatccatgctnagtan

SEQ ID NO: 19 - RNA, 21 nt, Synthetic Construct
  source 1..21: mol_type = other RNA; note = modified anti-sense strand; note (original language) = 经修饰的反义链; organism (original language) = 合成构建体
  modified_base 1: mod_base = OTHER; note = modified with 2'-methoxy; note (original language) = 2'-甲氧基修饰的
  modified_base 2: mod_base = OTHER; note = modified with 2'-Fluoro; note (original language) = 2'-氟代修饰的
  modified_base 3: mod_base = OTHER; note = modified with 2'-methoxy; note (original language) = 2'-甲氧基修饰的
  modified_base 4: mod_base = OTHER; note = modified with 2'-Fluoro; note (original language) = 2'-氟代修饰的
  modified_base 5: mod_base = OTHER; note = modified with 2'-methoxy; note (original language) = 2'-甲氧基修饰的
  modified_base 6: mod_base = OTHER; note = modified with 2'-Fluoro; note (original language) = 2'-氟代修饰的
  modified_base 7: mod_base = OTHER; note = modified with 2'-methoxy; note (original language) = 2'-甲氧基修饰的
  modified_base 8: mod_base = OTHER; note = modified with 2'-Fluoro; note (original language) = 2'-氟代修饰的
  modified_base 9: mod_base = OTHER; note = modified with 2'-methoxy; note (original language) = 2'-甲氧基修饰的
  modified_base 10: mod_base = OTHER; note = modified with 2'-Fluoro; note (original language) = 2'-氟代修饰的
  modified_base 11: mod_base = OTHER; note = modified with 2'-methoxy; note (original language) = 2'-甲氧基修饰的
  modified_base 12: mod_base = OTHER; note = modified with 2'-Fluoro; note (original language) = 2'-氟代修饰的
  modified_base 13: mod_base = OTHER; note = modified with 2'-methoxy; note (original language) = 2'-甲氧基修饰的
  modified_base 14: mod_base = OTHER; note = modified with 2'-Fluoro; note (original language) = 2'-氟代修饰的
  modified_base 15: mod_base = OTHER; note = modified with 2'-methoxy; note (original language) = 2'-甲氧基修饰的
  modified_base 16: mod_base = OTHER; note = modified with 2'-Fluoro; note (original language) = 2'-氟代修饰的
  modified_base 17: mod_base = OTHER; note = modified with 2'-methoxy; note (original language) = 2'-甲氧基修饰的
  modified_base 18: mod_base = OTHER; note = modified with 2'-Fluoro; note (original language) = 2'-氟代修饰的
  modified_base 19: mod_base = OTHER; note = modified with 2'-methoxy; note (original language) = 2'-甲氧基修饰的
  modified_base 20: mod_base = OTHER; note = modified with 2'-Fluoro; note (original language) = 2'-氟代修饰的
  modified_base 21: mod_base = OTHER; note = modified with 2'-methoxy; note (original language) = 2'-甲氧基修饰的
  modified_base 1..4: mod_base = OTHER; note = two adjacent nucleosides are linked by phosphorothioate diester groups; note (original language) = 相邻的两个核苷之间为硫代磷酸二酯基连接
  modified_base 20..21: mod_base = OTHER; note = two adjacent nucleosides are linked by phosphorothioate diester groups; note (original language) = 相邻的两个核苷之间为硫代磷酸二酯基连接
  modified_base 1: mod_base = OTHER; note = 5'-E-VP; note (original language) = 5'末端为反式-乙烯基磷酸二酯基
tactcagcatggatcatgtgg

SEQ ID NO: 20 - RNA, 22 nt, Synthetic Construct
  source 1..22: mol_type = other RNA; note = modified sense strand; note (original language) = 经修饰的正义链; organism (original language) = 合成构建体
  modified_base 22: mod_base = OTHER; note = n is a reverse reverse nucleotide without base modification; note (original language) = n为反向无碱基修饰的核苷
  modified_base 1..8: mod_base = OTHER; note = modified with 2'-methoxy; note (original language) = 2'-甲氧基修饰的
  modified_base 9..11: mod_base = OTHER; note = modified with 2'-Fluoro; note (original language) = 2'-氟代修饰的
  modified_base 12..21: mod_base = OTHER; note = modified with 2'-methoxy; note (original language) = 2'-甲氧基修饰的
  modified_base 1..2: mod_base = OTHER; note = two adjacent nucleosides are linked by phosphorothioate diester groups; note (original language) = 相邻的两个核苷之间为硫代磷酸二酯基连接
  modified_base 21..22: mod_base = OTHER; note = two adjacent nucleosides are linked by phosphorothioate diester groups; note (original language) = 相邻的两个核苷之间为硫代磷酸二酯基连接
  modified_base 1: mod_base = OTHER; note = the 5' end is conjugated with the targeting ligand III-5; note (original language) = 5'端与靶向配体III-5缀合
  modified_base 17: mod_base = OTHER; note = n is a hypoxanthine 2'-OMe riboside; note (original language) = n为次黄嘌呤2'-OMe核糖核苷
ccacatgatccatgctnagtan

SEQ ID NO: 21 - RNA, 22 nt, Synthetic Construct
  source 1..22: mol_type = other RNA; note = modified sense strand; note (original language) = 经修饰的正义链; organism (original language) = 合成构建体
  modified_base 17: mod_base = OTHER; note = n is a hypoxanthine 2'-OMe riboside; note (original language) = n为次黄嘌呤2'-OMe核糖核苷
  modified_base 22: mod_base = OTHER; note = n is a reverse reverse nucleotide without base modification; note (original language) = n为反向无碱基修饰的核苷
  modified_base 1..8: mod_base = OTHER; note = modified with 2'-methoxy; note (original language) = 2'-甲氧基修饰的
  modified_base 9..11: mod_base = OTHER; note = modified with 2'-Fluoro; note (original language) = 2'-氟代修饰的
  modified_base 12..21: mod_base = OTHER; note = modified with 2'-methoxy; note (original language) = 2'-甲氧基修饰的
  modified_base 1..2: mod_base = OTHER; note = two adjacent nucleosides are linked by phosphorothioate diester groups; note (original language) = 相邻的两个核苷之间为硫代磷酸二酯基连接
  modified_base 21..22: mod_base = OTHER; note = two adjacent nucleosides are linked by phosphorothioate diester groups; note (original language) = 相邻的两个核苷之间为硫代磷酸二酯基连接
  modified_base 1: mod_base = OTHER; note = the 5' end is conjugated with the targeting ligand III-3; note (original language) = 5'端与靶向配体III-3缀合
ccacatgatccatgctnagtan

SEQ ID NO: 22 - RNA, 22 nt, Synthetic Construct
  source 1..22: mol_type = other RNA; note = modified sense strand; note (original language) = 经修饰的正义链; organism (original language) = 合成构建体
  modified_base 17: mod_base = OTHER; note = n is a hypoxanthine 2'-OMe riboside; note (original language) = n为次黄嘌呤2'-OMe核糖核苷
  modified_base 22: mod_base = OTHER; note = n is a reverse reverse nucleotide without base modification; note (original language) = n为反向无碱基修饰的核苷
  modified_base 1..8: mod_base = OTHER; note = modified with 2'-methoxy; note (original language) = 2'-甲氧基修饰的
  modified_base 9..11: mod_base = OTHER; note = modified with 2'-Fluoro; note (original language) = 2'-氟代修饰的
  modified_base 12..21: mod_base = OTHER; note = modified with 2'-methoxy; note (original language) = 2'-甲氧基修饰的
  modified_base 1..2: mod_base = OTHER; note = two adjacent nucleosides are linked by phosphorothioate diester groups; note (original language) = 相邻的两个核苷之间为硫代磷酸二酯基连接
  modified_base 21..22: mod_base = OTHER; note = two adjacent nucleosides are linked by phosphorothioate diester groups; note (original language) = 相邻的两个核苷之间为硫代磷酸二酯基连接
  modified_base 1: mod_base = OTHER; note = the 5' end is conjugated with the targeting ligand III-2; note (original language) = 5'端与靶向配体III-2缀合
ccacatgatccatgctnagtan

SEQ ID NO: 23 - RNA, 22 nt, Synthetic Construct
  source 1..22: mol_type = other RNA; note = modified sense strand; note (original language) = 经修饰的正义链; organism (original language) = 合成构建体
  modified_base 17: mod_base = OTHER; note = n is a hypoxanthine 2'-OMe riboside; note (original language) = n为次黄嘌呤2'-OMe核糖核苷
  modified_base 22: mod_base = OTHER; note = n is a reverse reverse nucleotide without base modification; note (original language) = n为反向无碱基修饰的核苷
  modified_base 1..8: mod_base = OTHER; note = modified with 2'-methoxy; note (original language) = 2'-甲氧基修饰的
  modified_base 9..11: mod_base = OTHER; note = modified with 2'-Fluoro; note (original language) = 2'-氟代修饰的
  modified_base 12..21: mod_base = OTHER; note = modified with 2'-methoxy; note (original language) = 2'-甲氧基修饰的
  modified_base 1..2: mod_base = OTHER; note = two adjacent nucleosides are linked by phosphorothioate diester groups; note (original language) = 相邻的两个核苷之间为硫代磷酸二酯基连接
  modified_base 21..22: mod_base = OTHER; note = two adjacent nucleosides are linked by phosphorothioate diester groups; note (original language) = 相邻的两个核苷之间为硫代磷酸二酯基连接
  modified_base 1: mod_base = OTHER; note = the 5' end is conjugated with the targeting ligand III-S1113-8; note (original language) = 5'端与靶向配体III-S1113-8缀合
ccacatgatccatgctnagtan

SEQ ID NO: 24 - RNA, 22 nt, Synthetic Construct
  source 1..22: mol_type = other RNA; note = modified sense strand; note (original language) = 经修饰的正义链; organism (original language) = 合成构建体
  modified_base 17: mod_base = OTHER; note = n is a hypoxanthine 2'-OMe riboside; note (original language) = n为次黄嘌呤2'-OMe核糖核苷
  modified_base 22: mod_base = OTHER; note = n is a reverse reverse nucleotide without base modification; note (original language) = n为反向无碱基修饰的核苷
  modified_base 1..8: mod_base = OTHER; note = modified with 2'-methoxy; note (original language) = 2'-甲氧基修饰的
  modified_base 9..11: mod_base = OTHER; note = modified with 2'-Fluoro; note (original language) = 2'-氟代修饰的
  modified_base 12..21: mod_base = OTHER; note = modified with 2'-methoxy; note (original language) = 2'-甲氧基修饰的
  modified_base 1..2: mod_base = OTHER; note = two adjacent nucleosides are linked by phosphorothioate diester groups; note (original language) = 相邻的两个核苷之间为硫代磷酸二酯基连接
  modified_base 21..22: mod_base = OTHER; note = two adjacent nucleosides are linked by phosphorothioate diester groups; note (original language) = 相邻的两个核苷之间为硫代磷酸二酯基连接
  modified_base 1: mod_base = OTHER; note = the 5' end is conjugated with the targeting ligand III-S1113-11; note (original language) = 5'端与靶向配体III-S1113-11缀合
ccacatgatccatgctnagtan

SEQ ID NO: 25 - RNA, 22 nt, Synthetic Construct
  source 1..22: mol_type = other RNA; note = modified sense strand; note (original language) = 经修饰的正义链; organism (original language) = 合成构建体
  modified_base 17: mod_base = OTHER; note = n is a hypoxanthine 2'-OMe riboside; note (original language) = n为次黄嘌呤2'-OMe核糖核苷
  modified_base 22: mod_base = OTHER; note = n is a reverse reverse nucleotide without base modification; note (original language) = n为反向无碱基修饰的核苷
  modified_base 1..8: mod_base = OTHER; note = modified with 2'-methoxy; note (original language) = 2'-甲氧基修饰的
  modified_base 9..11: mod_base = OTHER; note = modified with 2'-Fluoro; note (original language) = 2'-氟代修饰的
  modified_base 12..21: mod_base = OTHER; note = modified with 2'-methoxy; note (original language) = 2'-甲氧基修饰的
  modified_base 1..2: mod_base = OTHER; note = two adjacent nucleosides are linked by phosphorothioate diester groups; note (original language) = 相邻的两个核苷之间为硫代磷酸二酯基连接
  modified_base 21..22: mod_base = OTHER; note = two adjacent nucleosides are linked by phosphorothioate diester groups; note (original language) = 相邻的两个核苷之间为硫代磷酸二酯基连接
  modified_base 1: mod_base = OTHER; note = the 5' end is conjugated with the targeting ligand III-S1113-13; note (original language) = 5'端与靶向配体III-S1113-13缀合
ccacatgatccatgctnagtan

SEQ ID NO: 26 - RNA, 22 nt, Synthetic Construct
  source 1..22: mol_type = other RNA; note = modified sense strand; note (original language) = 经修饰的正义链; organism (original language) = 合成构建体
  modified_base 17: mod_base = OTHER; note = n is a hypoxanthine 2'-OMe riboside; note (original language) = n为次黄嘌呤2'-OMe核糖核苷
  modified_base 22: mod_base = OTHER; note = n is a reverse reverse nucleotide without base modification; note (original language) = n为反向无碱基修饰的核苷
  modified_base 1..8: mod_base = OTHER; note = modified with 2'-methoxy; note (original language) = 2'-甲氧基修饰的
  modified_base 9..11: mod_base = OTHER; note = modified with 2'-Fluoro; note (original language) = 2'-氟代修饰的
  modified_base 12..21: mod_base = OTHER; note = modified with 2'-methoxy; note (original language) = 2'-甲氧基修饰的
  modified_base 1..2: mod_base = OTHER; note = two adjacent nucleosides are linked by phosphorothioate diester groups; note (original language) = 相邻的两个核苷之间为硫代磷酸二酯基连接
  modified_base 21..22: mod_base = OTHER; note = two adjacent nucleosides are linked by phosphorothioate diester groups; note (original language) = 相邻的两个核苷之间为硫代磷酸二酯基连接
  modified_base 1: mod_base = OTHER; note = the 5' end is conjugated with the targeting ligand TA14''; note (original language) = 5'端与靶向配体TA14''缀合
ccacatgatccatgctnagtan

SEQ ID NO: 27 - RNA, 22 nt, Synthetic Construct
  source 1..22: mol_type = other RNA; note = modified sense strand; note (original language) = 经修饰的正义链; organism (original language) = 合成构建体
  modified_base 22: mod_base = OTHER; note = n is a reverse reverse nucleotide without base modification; note (original language) = n为反向无碱基修饰的核苷
  modified_base 1..6: mod_base = OTHER; note = modified with 2'-methoxy; note (original language) = 2'-甲氧基修饰的
  modified_base 7: mod_base = OTHER; note = modified with 2'-Fluoro; note (original language) = 2'-氟代修饰的
  modified_base 8: mod_base = OTHER; note = modified with 2'-methoxy; note (original language) = 2'-甲氧基修饰的
  modified_base 9..11: mod_base = OTHER; note = modified with 2'-Fluoro; note (original language) = 2'-氟代修饰的
  modified_base 12..21: mod_base = OTHER; note = modified with 2'-methoxy; note (original language) = 2'-甲氧基修饰的
  modified_base 1..3: mod_base = OTHER; note = two adjacent nucleosides are linked by phosphorothioate diester groups; note (original language) = 相邻的两个核苷之间为硫代磷酸二酯基连接
  modified_base 20..22: mod_base = OTHER; note = two adjacent nucleosides are linked by phosphorothioate diester groups; note (original language) = 相邻的两个核苷之间为硫代磷酸二酯基连接
  modified_base 1: mod_base = OTHER; note = the 5' end is conjugated with the targeting ligand III-S1113-8; note (original language) = 5'端与靶向配体III-S1113-8缀合
gtgctttaactacaatatacan

SEQ ID NO: 28 - RNA, 23 nt, Synthetic Construct
  source 1..23: mol_type = other RNA; note = modified anti-sense strand; note (original language) = 经修饰的反义链; organism (original language) = 合成构建体
  modified_base 1: mod_base = OTHER; note = modified with 2'-methoxy; note (original language) = 2'-甲氧基修饰的
  modified_base 2: mod_base = OTHER; note = modified with 2'-Fluoro; note (original language) = 2'-氟代修饰的
  modified_base 3..5: mod_base = OTHER; note = modified with 2'-methoxy; note (original language) = 2'-甲氧基修饰的
  modified_base 6: mod_base = OTHER; note = modified with 2'-Fluoro; note (original language) = 2'-氟代修饰的
  modified_base 7: mod_base = OTHER; note = modified with 2'-methoxy; note (original language) = 2'-甲氧基修饰的
  modified_base 8..9: mod_base = OTHER; note = modified with 2'-Fluoro; note (original language) = 2'-氟代修饰的
  modified_base 10..13: mod_base = OTHER; note = modified with 2'-methoxy; note (original language) = 2'-甲氧基修饰的
  modified_base 14: mod_base = OTHER; note = modified with 2'-Fluoro; note (original language) = 2'-氟代修饰的
  modified_base 15: mod_base = OTHER; note = modified with 2'-methoxy; note (original language) = 2'-甲氧基修饰的
  modified_base 16: mod_base = OTHER; note = modified with 2'-Fluoro; note (original language) = 2'-氟代修饰的
  modified_base 17..23: mod_base = OTHER; note = modified with 2'-methoxy; note (original language) = 2'-甲氧基修饰的
  modified_base 1..3: mod_base = OTHER; note = two adjacent nucleosides are linked by phosphorothioate diester groups; note (original language) = 相邻的两个核苷之间为硫代磷酸二酯基连接
  modified_base 1: mod_base = OTHER; note = 5'-E-VP; note (original language) = 5'末端为反式-乙烯基磷酸二酯基
  modified_base 21..23: mod_base = OTHER; note = two adjacent nucleosides are linked by phosphorothioate diester groups; note (original language) = 相邻的两个核苷之间为硫代磷酸二酯基连
tgtatattgtagttaaagcacat

SEQ ID NO: 29 - RNA, 22 nt, Synthetic Construct
  source 1..22: mol_type = other RNA; note = modified sense strand; note (original language) = 经修饰的正义链; organism (original language) = 合成构建体
  modified_base 1..6: mod_base = OTHER; note = modified with 2'-methoxy; note (original language) = 2'-甲氧基修饰的
  modified_base 7: mod_base = OTHER; note = modified with 2'-Fluoro; note (original language) = 2'-氟代修饰的
  modified_base 8: mod_base = OTHER; note = modified with 2'-methoxy; note (original language) = 2'-甲氧基修饰的
  modified_base 9..11: mod_base = OTHER; note = modified with 2'-Fluoro; note (original language) = 2'-氟代修饰的
  modified_base 12..21: mod_base = OTHER; note = modified with 2'-methoxy; note (original language) = 2'-甲氧基修饰的
  modified_base 22: mod_base = OTHER; note = n is a reverse reverse nucleotide without base modification; note (original language) = n为反向无碱基修饰的核苷
  modified_base 1..3: mod_base = OTHER; note = two adjacent nucleosides are linked by phosphorothioate diester groups; note (original language) = 相邻的两个核苷之间为硫代磷酸二酯基连接
  modified_base 20..22: mod_base = OTHER; note = two adjacent nucleosides are linked by phosphorothioate diester groups; note (original language) = 相邻的两个核苷之间为硫代磷酸二酯基连接
  modified_base 1: mod_base = OTHER; note = the 5' end is conjugated with the targeting ligand III-S1113-11; note (original language) = 5'端与靶向配体III-S1113-11缀合
gtgctttaactacaatatacan

SEQ ID NO: 30 - RNA, 22 nt, Synthetic Construct
  source 1..22: mol_type = other RNA; note = modified sense strand; note (original language) = 经修饰的正义链; organism (original language) = 合成构建体
  modified_base 1..6: mod_base = OTHER; note = modified with 2'-methoxy; note (original language) = 2'-甲氧基修饰的
  modified_base 7: mod_base = OTHER; note = modified with 2'-Fluoro; note (original language) = 2'-氟代修饰的
  modified_base 8: mod_base = OTHER; note = modified with 2'-methoxy; note (original language) = 2'-甲氧基修饰的
  modified_base 9..11: mod_base = OTHER; note = modified with 2'-Fluoro; note (original language) = 2'-氟代修饰的
  modified_base 12..21: mod_base = OTHER; note = modified with 2'-methoxy; note (original language) = 2'-甲氧基修饰的
  modified_base 22: mod_base = OTHER; note = n is a reverse reverse nucleotide without base modification; note (original language) = n为反向无碱基修饰的核苷
  modified_base 1..3: mod_base = OTHER; note = two adjacent nucleosides are linked by phosphorothioate diester groups; note (original language) = 相邻的两个核苷之间为硫代磷酸二酯基连接
  modified_base 20..22: mod_base = OTHER; note = two adjacent nucleosides are linked by phosphorothioate diester groups; note (original language) = 相邻的两个核苷之间为硫代磷酸二酯基连接
  modified_base 1: mod_base = OTHER; note = the 5' end is conjugated with the targeting ligand III-S1113-13; note (original language) = 5'端与靶向配体III-S1113-13缀合
gtgctttaactacaatatacan

SEQ ID NO: 31 - RNA, 22 nt, Synthetic Construct
  source 1..22: mol_type = other RNA; note = modified sense strand; note (original language) = 经修饰的正义链; organism (original language) = 合成构建体
  modified_base 22: mod_base = OTHER; note = n is a reverse reverse nucleotide without base modification; note (original language) = n为反向无碱基修饰的核苷
  modified_base 1..6: mod_base = OTHER; note = modified with 2'-methoxy; note (original language) = 2'-甲氧基修饰的
  modified_base 7: mod_base = OTHER; note = modified with 2'-Fluoro; note (original language) = 2'-氟代修饰的
  modified_base 8: mod_base = OTHER; note = modified with 2'-methoxy; note (original language) = 2'-甲氧基修饰的
  modified_base 9..11: mod_base = OTHER; note = modified with 2'-Fluoro; note (original language) = 2'-氟代修饰的
  modified_base 12..21: mod_base = OTHER; note = modified with 2'-methoxy; note (original language) = 2'-甲氧基修饰的
  modified_base 1..3: mod_base = OTHER; note = two adjacent nucleosides are linked by phosphorothioate diester groups; note (original language) = 相邻的两个核苷之间为硫代磷酸二酯基连接
  modified_base 20..22: mod_base = OTHER; note = two adjacent nucleosides are linked by phosphorothioate diester groups; note (original language) = 相邻的两个核苷之间为硫代磷酸二酯基连接
  modified_base 1: mod_base = OTHER; note = the 5' end is conjugated with the targeting ligand TA14''; note (original language) = 5'端与靶向配体TA14''缀合
gtgctttaactacaatatacan

SEQ ID NO: 32 - RNA, 22 nt, Synthetic Construct
  source 1..22: mol_type = other RNA; organism (original language) = 合成构建体
  modified_base 22: mod_base = OTHER; note = n is a reverse reverse nucleotide without base modification; note (original language) = n为反向无碱基修饰的核苷
  modified_base 1..6: mod_base = OTHER; note = modified with 2'-methoxy; note (original language) = 2'-甲氧基修饰的
  modified_base 7: mod_base = OTHER; note = modified with 2'-Fluoro; note (original language) = 2'-氟代修饰的
  modified_base 8: mod_base = OTHER; note = modified with 2'-methoxy; note (original language) = 2'-甲氧基修饰的
  modified_base 9..11: mod_base = OTHER; note = modified with 2'-Fluoro; note (original language) = 2'-氟代修饰的
  modified_base 12..21: mod_base = OTHER; note = modified with 2'-methoxy; note (original language) = 2'-甲氧基修饰的
  modified_base 1..3: mod_base = OTHER; note = two adjacent nucleosides are linked by phosphorothioate diester groups; note (original language) = 相邻的两个核苷之间为硫代磷酸二酯基连接
  modified_base 20..22: mod_base = OTHER; note = two adjacent nucleosides are linked by phosphorothioate diester groups; note (original language) = 相邻的两个核苷之间为硫代磷酸二酯基连接
  modified_base 1: mod_base = OTHER; note = the 5' end is conjugated with the targeting ligand III-3; note (original language) = 5'端与靶向配体III-3缀合
gtgctttaactacaatatacan

SEQ ID NO: 33 - RNA, 22 nt, Synthetic Construct
  source 1..22: mol_type = other RNA; note = modified sense strand; note (original language) = 经修饰的正义链; organism (original language) = 合成构建体
  modified_base 22: mod_base = OTHER; note = n is a reverse reverse nucleotide without base modification; note (original language) = n为反向无碱基修饰的核苷
  modified_base 1..6: mod_base = OTHER; note = modified with 2'-methoxy; note (original language) = 2'-甲氧基修饰的
  modified_base 7: mod_base = OTHER; note = modified with 2'-Fluoro; note (original language) = 2'-氟代修饰的
  modified_base 8: mod_base = OTHER; note = modified with 2'-methoxy; note (original language) = 2'-甲氧基修饰的
  modified_base 9..11: mod_base = OTHER; note = modified with 2'-Fluoro; note (original language) = 2'-氟代修饰的
  modified_base 12..21: mod_base = OTHER; note = modified with 2'-methoxy; note (original language) = 2'-甲氧基修饰的
  modified_base 1..3: mod_base = OTHER; note = two adjacent nucleosides are linked by phosphorothioate diester groups; note (original language) = 相邻的两个核苷之间为硫代磷酸二酯基连接
  modified_base 20..22: mod_base = OTHER; note = two adjacent nucleosides are linked by phosphorothioate diester groups; note (original language) = 相邻的两个核苷之间为硫代磷酸二酯基连接
  modified_base 1: mod_base = OTHER; note = the 5' end is conjugated with the targeting ligand III-2; note (original language) = 5'端与靶向配体III-2缀合
gtgctttaactacaatatacan

SEQ ID NO: 34 - RNA, 22 nt, Synthetic Construct
  source 1..22: mol_type = other RNA; note = modified sense strand; note (original language) = 经修饰的正义链; organism (original language) = 合成构建体
  modified_base 22: mod_base = OTHER; note = n is a reverse reverse nucleotide without base modification; note (original language) = n为反向无碱基修饰的核苷
  modified_base 1..6: mod_base = OTHER; note = modified with 2'-methoxy; note (original language) = 2'-甲氧基修饰的
  modified_base 7: mod_base = OTHER; note = modified with 2'-Fluoro; note (original language) = 2'-氟代修饰的
  modified_base 8: mod_base = OTHER; note = modified with 2'-methoxy; note (original language) = 2'-甲氧基修饰的
  modified_base 9..11: mod_base = OTHER; note = modified with 2'-Fluoro; note (original language) = 2'-氟代修饰的
  modified_base 12..21: mod_base = OTHER; note = modified with 2'-methoxy; note (original language) = 2'-甲氧基修饰的
  modified_base 1..3: mod_base = OTHER; note = two adjacent nucleosides are linked by phosphorothioate diester groups; note (original language) = 相邻的两个核苷之间为硫代磷酸二酯基连接
  modified_base 20..22: mod_base = OTHER; note = two adjacent nucleosides are linked by phosphorothioate diester groups; note (original language) = 相邻的两个核苷之间为硫代磷酸二酯基连接
  modified_base 1: mod_base = OTHER; note = the 5' end is conjugated with the targeting ligand III-5; note (original language) = 5'端与靶向配体III-5缀合
gtgctttaactacaatatacan

SEQ ID NO: 35 - RNA, 22 nt, Synthetic Construct
  source 1..22: mol_type = other RNA; note = modified sense strand; note (original language) = 经修饰的正义链; organism (original language) = 合成构建体
  modified_base 1..6: mod_base = OTHER; note = modified with 2'-methoxy; note (original language) = 2'-甲氧基修饰的
  modified_base 22: mod_base = OTHER; note = n is a reverse reverse nucleotide without base modification; note (original language) = n为反向无碱基修饰的核苷
  modified_base 7: mod_base = OTHER; note = modified with 2'-Fluoro; note (original language) = 2'-氟代修饰的
  modified_base 8: mod_base = OTHER; note = modified with 2'-methoxy; note (original language) = 2'-甲氧基修饰的
  modified_base 9..11: mod_base = OTHER; note = modified with 2'-Fluoro; note (original language) = 2'-氟代修饰的
  modified_base 12..21: mod_base = OTHER; note = modified with 2'-methoxy; note (original language) = 2'-甲氧基修饰的
  modified_base 1..3: mod_base = OTHER; note = two adjacent nucleosides are linked by phosphorothioate diester groups; note (original language) = 相邻的两个核苷之间为硫代磷酸二酯基连接
  modified_base 20..22: mod_base = OTHER; note = two adjacent nucleosides are linked by phosphorothioate diester groups; note (original language) = 相邻的两个核苷之间为硫代磷酸二酯基连接
  modified_base 1: mod_base = OTHER; note = the 5' end is conjugated with the targeting ligand III-S1113-8; note (original language) = 5'端与靶向配体III-S1113-8缀合
ccggtcccaggttatgacacan

SEQ ID NO: 36 - RNA, 23 nt, Synthetic Construct
  source 1..23: mol_type = other RNA; note = modified anti-sense strand; note (original language) = 经修饰的反义链; organism (original language) = 合成构建体
  modified_base 1: mod_base = OTHER; note = modified with 2'-methoxy; note (original language) = 2'-甲氧基修饰的
  modified_base 2: mod_base = OTHER; note = modified with 2'-Fluoro; note (original language) = 2'-氟代修饰的
  modified_base 3..5: mod_base = OTHER; note = modified with 2'-methoxy; note (original language) = 2'-甲氧基修饰的
  modified_base 6: mod_base = OTHER; note = modified with 2'-Fluoro; note (original language) = 2'-氟代修饰的
  modified_base 7: mod_base = OTHER; note = modified with 2'-methoxy; note (original language) = 2'-甲氧基修饰的
  modified_base 8..9: mod_base = OTHER; note = modified with 2'-Fluoro; note (original language) = 2'-氟代修饰的
  modified_base 10..13: mod_base = OTHER; note = modified with 2'-methoxy; note (original language) = 2'-甲氧基修饰的
  modified_base 14: mod_base = OTHER; note = modified with 2'-Fluoro; note (original language) = 2'-氟代修饰的
  modified_base 15: mod_base = OTHER; note = modified with 2'-methoxy; note (original language) = 2'-甲氧基修饰的
  modified_base 16: mod_base = OTHER; note = modified with 2'-Fluoro; note (original language) = 2'-氟代修饰的
  modified_base 17..23: mod_base = OTHER; note = modified with 2'-methoxy; note (original language) = 2'-甲氧基修饰的
  modified_base 1..3: mod_base = OTHER; note = two adjacent nucleosides are linked by phosphorothioate diester groups; note (original language) = 相邻的两个核苷之间为硫代磷酸二酯基连接
  modified_base 21..23: mod_base = OTHER; note = two adjacent nucleosides are linked by phosphorothioate diester groups; note (original language) = 相邻的两个核苷之间为硫代磷酸二酯基连接
  modified_base 1: mod_base = OTHER; note = 5'-E-VP; note (original language) = 5'末端为反式-乙烯基磷酸二酯基
tgtgtcataacctgggaccggat

SEQ ID NO: 37 - RNA, 22 nt, Synthetic Construct
  source 1..22: mol_type = other RNA; note = modified sense strand; note (original language) = 经修饰的正义链; organism (original language) = 合成构建体
  modified_base 22: mod_base = OTHER; note = n is a reverse reverse nucleotide without base modification; note (original language) = n为反向无碱基修饰的核苷
  modified_base 1..6: mod_base = OTHER; note = modified with 2'-methoxy; note (original language) = 2'-甲氧基修饰的
  modified_base 7: mod_base = OTHER; note = modified with 2'-Fluoro; note (original language) = 2'-氟代修饰的
  modified_base 8: mod_base = OTHER; note = modified with 2'-methoxy; note (original language) = 2'-甲氧基修饰的
  modified_base 9..11: mod_base = OTHER; note = modified with 2'-Fluoro; note (original language) = 2'-氟代修饰的
  modified_base 12..21: mod_base = OTHER; note = modified with 2'-methoxy; note (original language) = 2'-甲氧基修饰的
  modified_base 1..3: mod_base = OTHER; note = two adjacent nucleosides are linked by phosphorothioate diester groups; note (original language) = 相邻的两个核苷之间为硫代磷酸二酯基连接
  modified_base 20..22: mod_base = OTHER; note = two adjacent nucleosides are linked by phosphorothioate diester groups; note (original language) = 相邻的两个核苷之间为硫代磷酸二酯基连接
  modified_base 1: mod_base = OTHER; note = the 5' end is conjugated with the targeting ligand III-S1113-11; note (original language) = 5'端与靶向配体III-S1113-11缀合
ccggtcccaggttatgacacan

SEQ ID NO: 38 - RNA, 22 nt, Synthetic Construct
  source 1..22: mol_type = other RNA; note = modified sense strand; note (original language) = 经修饰的正义链; organism (original language) = 合成构建体
  modified_base 22: mod_base = OTHER; note = n is a reverse reverse nucleotide without base modification; note (original language) = n为反向无碱基修饰的核苷
  modified_base 1..6: mod_base = OTHER; note = modified with 2'-methoxy; note (original language) = 2'-甲氧基修饰的
  modified_base 7: mod_base = OTHER; note = modified with 2'-Fluoro; note (original language) = 2'-氟代修饰的
  modified_base 8: mod_base = OTHER; note = modified with 2'-methoxy; note (original language) = 2'-甲氧基修饰的
  modified_base 9..11: mod_base = OTHER; note = modified with 2'-Fluoro; note (original language) = 2'-氟代修饰的
  modified_base 12..21: mod_base = OTHER; note = modified with 2'-methoxy; note (original language) = 2'-甲氧基修饰的
  modified_base 1..3: mod_base = OTHER; note = two adjacent nucleosides are linked by phosphorothioate diester groups; note (original language) = 相邻的两个核苷之间为硫代磷酸二酯基连接
  modified_base 20..22: mod_base = OTHER; note = two adjacent nucleosides are linked by phosphorothioate diester groups; note (original language) = 相邻的两个核苷之间为硫代磷酸二酯基连接
  modified_base 1: mod_base = OTHER; note = the 5' end is conjugated with the targeting ligand III-S1113-13; note (original language) = 5'端与靶向配体III-S1113-13缀合
ccggtcccaggttatgacacan

SEQ ID NO: 39 - DNA, 21 bp, Synthetic Construct
  source 1..21: PCR_primers = fwd_name: RAGE, fwd_seq: ttgagcctgaaggtggaatag,rev_name: RAGE, rev_seq: agggtgcaccatcctttatc; mol_type = other DNA; organism (original language) = 合成构建体
ttgagcctgaaggtggaatag

SEQ ID NO: 40 - DNA, 20 bp, Synthetic Construct
  source 1..20: PCR_primers = fwd_name: RAGE, fwd_seq: ttgagcctgaaggtggaatag,rev_name: RAGE, rev_seq: agggtgcaccatcctttatc; mol_type = other DNA; organism (original language) = 合成构建体
agggtgcaccatcctttatc

SEQ ID NO: 41 - DNA, 25 bp, Synthetic Construct
  source 1..25: mol_type = other DNA; note = RAGE-Probe; organism (original language) = 合成构建体
cagagatggcacaggtcaaggtcac

SEQ ID NO: 42 - DNA, 20 bp, Synthetic Construct
  source 1..20: PCR_primers = fwd_name: GAPDH, fwd_seq: aacagcaactcccactcttc,rev_name: GAPDH, rev_seq: cctgttgctgtagccgtatt; mol_type = other DNA; organism (original language) = 合成构建体
aacagcaactcccactcttc

SEQ ID NO: 43 - DNA, 20 bp, Synthetic Construct
  source 1..20: PCR_primers = fwd_name: GAPDH, fwd_seq: aacagcaactcccactcttc,rev_name: GAPDH, rev_seq: cctgttgctgtagccgtatt; mol_type = other DNA; organism (original language) = 合成构建体
cctgttgctgtagccgtatt

SEQ ID NO: 44 - DNA, 27 bp, Synthetic Construct
  source 1..27: mol_type = other DNA; note = GAPDH-Probe; organism (original language) = 合成构建体
aaagttgtcattgagagcaatgccagc

SEQ ID NO: 45 - DNA, 22 bp, Synthetic Construct
  source 1..22: PCR_primers = fwd_name: MUC5B, fwd_seq: aggtgctctgttgtagtgttag,rev_name: MUC5B, rev_seq: gtgttgggaagaggcatagaa; mol_type = other DNA; organism (original language) = 合成构建体
aggtgctctgttgtagtgttag

SEQ ID NO: 46 - DNA, 21 bp, Synthetic Construct
  source 1..21: PCR_primers = fwd_name: MUC5B, fwd_seq: aggtgctctgttgtagtgttag,rev_name: MUC5B, rev_seq: gtgttgggaagaggcatagaa; mol_type = other DNA; organism (original language) = 合成构建体
gtgttgggaagaggcatagaa

SEQ ID NO: 47 - DNA, 27 bp, Synthetic Construct
  source 1..27: mol_type = other DNA; note = MUC5B-Probe; organism (original language) = 合成构建体
caatgacaggatcagcaactactgcca

SEQ ID NO: 48 - DNA, 20 bp, Synthetic Construct
  source 1..20: PCR_primers = fwd_name: GAPDH, fwd_seq: aacagcaactcccactcttc,rev_name: GAPDH, rev_seq: cctgttgctgtagccgtatt; mol_type = other DNA
aacagcaactcccactcttc

SEQ ID NO: 49 - DNA, 20 bp, Synthetic Construct
  source 1..20: PCR_primers = fwd_name: GAPDH, fwd_seq: aacagcaactcccactcttc,rev_name: GAPDH, rev_seq: cctgttgctgtagccgtatt; mol_type = other DNA; organism (original language) = 合成构建体
cctgttgctgtagccgtatt

SEQ ID NO: 50 - DNA, 27 bp, Synthetic Construct
  source 1..27: mol_type = other DNA; note = GAPDH-Probe; organism (original language) = 合成构建体
aaagttgtcattgagagcaatgccagc

SEQ ID NO: 51 - DNA, 20 bp, Synthetic Construct
  source 1..20: PCR_primers = fwd_name: APP, fwd_seq: gacagacagcacaccctaaa,rev_name: APP, rev_seq: cacacggaggtgtgtcataa; mol_type = other DNA; organism (original language) = 合成构建体
gacagacagcacaccctaaa

SEQ ID NO: 52 - DNA, 20 bp, Synthetic Construct
  source 1..20: PCR_primers = fwd_name: APP, fwd_seq: gacagacagcacaccctaaa,rev_name: APP, rev_seq: cacacggaggtgtgtcataa; mol_type = other DNA; organism (original language) = 合成构建体
cacacggaggtgtgtcataa

SEQ ID NO: 53 - DNA, 24 bp, Synthetic Construct
  source 1..24: mol_type = other DNA; note = APP-Probe; organism (original language) = 合成构建体
atcccaagaaagccgctcagatcc

SEQ ID NO: 54 - DNA, 22 bp, Synthetic Construct
  source 1..22: PCR_primers = fwd_name: GAPDH, fwd_seq: ccaggtggtctcctctgacttc,rev_name: GAPDH, rev_seq: gtggtcgttgagggcaatg; mol_type = other DNA
ccaggtggtctcctctgacttc

SEQ ID NO: 55 - DNA, 19 bp, Synthetic Construct
  source 1..19: PCR_primers = fwd_name: GAPDH, fwd_seq: ccaggtggtctcctctgacttc,rev_name: GAPDH, rev_seq: gtggtcgttgagggcaatg; mol_type = other DNA; organism (original language) = 合成构建体
gtggtcgttgagggcaatg

SEQ ID NO: 56 - DNA, 25 bp, Synthetic Construct
  source 1..25: mol_type = other DNA; note = GAPDH-Probe; organism (original language) = 合成构建体
acagcgacacccactcctccacctt